European Patent Specification EP 4 069 729 B1, published January 22, 2025. Title: OPTIMIZED ENGINEERED MEGANUCLEASES HAVING SPECIFICITY FOR A RECOGNITION SEQUENCE IN THE HEPATITIS B VIRUS GENOME. Applicant: Precision BioSciences, Inc. Application Not Yet Assigned. The sequence listing filed with the application follows.

SEQUENCE LISTING (51 sequences)

SEQ ID NO: 1 - protein, 163 aa, Chlamydomonas reinhardtii
MNTKYNKEFLLYLAGFVDGDGSIIAQIKPNQSYKFKHQLSLAFQVTQKTQRRWFLDKLVDEIGVGYVRDRGSVSDYILSEIKPLHNFLTQLQPFLKLKQKQANLVLKIIWRLPSAKESPDKFLEVCTWVDQIAALNDSKTRKTTSETVRAVLDSLSEKKKSSP

SEQ ID NO: 2 - protein, 9 aa, Chlamydomonas reinhardtii
LAGLIDADG

SEQ ID NO: 3 - DNA, 3221 bp, Hepatitis B virus
ttccactgccttccaccaagctctgcaggatcccagagtcaggggtctgtattttcctgctggtggctccagttcaggaacagtaaaccctgctccgaatattgcctctcacatctcgtcaatctccgcgaggactggggaccctgtggcgaacatggagaacatcacatcaggattcctaggacccctgctcgtgttacaggcggggtttttcttgttgacaagaatcctcacaataccgcagagtctagactcgtggtggacttctctcaattttctagggggatcacccgtgtgtcttggccaaaattcgcagtccccaacctccaatcactcaccaacctcctgtcctccaatttgtcctggttatcgctggatgtgtctgcggcgttttatcatattcctcttcatcctgctgctatgcctcatcttcttattggttcttctggattatcaaggtatgttgcccgtttgtcctctaattccaggatcaacaacaaccagtacgggaccatgcaaaacctgcacgactcctgctcaaggcaactctatgtttccctcatgttgctgtacaaaacctacggatggaaattgcacctgtattcccatcccatcgtcctgggctttcgcaaaatacctatgggagtgggcctcagtccgtttctcttggctcagtttactagtgccatttgttcagtggttcgtagggctttcccccactgtttggctttcagctatatggatgatgtggtattgggggccaagtctgtacagcatcgtgagtccctttataccgctgttaccaattttcttttgtctctgggtatacatttaaaccctaacaaaacaaaaagatggggttattccctaaacttcatgggttacataattggaagttggggaactttgccacaggatcatattgtacaaaagatcaaacactgttttagaaaacttcctgttaacaggcctattgattggaaagtatgtcaaagaattgtgggtcttttgggctttgctgctccatttacacaatgtggatatcctgccttaatgcctttgtatgcatgtatacaagctaaacaggctttcactttctcgccaacttacaaggcctttctaagtaaacagtacatgaacctttaccccgttgctcggcaacggcctggtctgtgccaagtgtttgctgacgcaacccccactggctggggcttggccataggccatcagcgcatgcgtggaacctttgtggctcctctgccgatccatactgcggaactcctagccgcttgttttgctcgcagccggtctggagcaaagctcatcggaactgacaattctgtcgtcctctcgcggaaatatacatcgtttccatggctgctaggctgtgctgccaactggatccttcgcggaacgtcctttgtctacgtcccgtcggcgctgaatcccgcggacgacccctctcggggccgcttgggactctctcgtccccttctccgtctgccgttccagccgaccacggggcgcacctctctttacgcggtctccccgtctgtgccttctcatctgccggtccgtgtgcacttcgcttcacctctgcacgttgcatggagaccaccgtgaacgcccatcagatcctgcccaaggtcttacataagaggactcttggactcccagcaatgtcaacgaccgaccttgaggcctacttcaaagactgtgtgtttaaggactgggaggagctgggggaggagattaggttaaaggtctttgtattaggaggctgtaggcataaattggtctgcgcaccagcaccatgcaactttttcacctctgcctaatcatctcttgtacatgtcccactgttcaagcctccaagctgtgccttgggtggctttggggcatggacattgacccttataaagaatttggagctactgtggagttactctcgtttttgccttctgacttctttccttccgtcagagatctcctagacaccgcctcagctctgtatcgagaagccttagagtctcctgagcattgctcacctcaccatactgcactcaggcaagccattctctgctggggggaattgatgactctagctacctgggtgggtaataatttggaagatccagcatccagggatctagtagtcaattatgttaatactaacatgggtttaaagatcaggcaactattgtggtttcatatatcttgccttacttttggaagagagactgtacttgaatatttggtctctttcggagtgtggattcgcactcctccagcctatagaccaccaaatgcccctatcttatcaacaattccggaaactactgttgttagacgacgggaccgaggcaggtcccctagaagaagaactccctcgcctcgcagacgcagatctcaatcgccgcgtcgcagaagatctcaatctcgggaatctcaatgttagtattccttggactcataaggtgggaaactttacggggctttattcctctacagtacctatctttaatcctgaatggcaaactccttcctttcctaagattcatttacaagaggacattattaataggtgtcaacaatttgtgggccctctcactgtaaatgaaaagagaagattgaaattaattatgcctgctagattctatcctacccacactaaatatttgcccttagacaaaggaattaaaccttattatccagatcaggtagttaatcattacttccaaaccagacattatttacatactctttggaaggctggtattctatataagagggaaaccacacgtagcgcatcattttgcgggtcaccatattcttgggaacaagagctacagcatgggaggttggtcatcaaaacctcgcaaaggcatggggacgaatctttctgttcccaaccctctgggattctttcccgatcatcagttggaccctgcattcggagccaactcaaacaatccagattgggacttcaaccccatcaaggaccactggccaacagccaaccaggtaggagtgggagcattcgggccagggctcacccctccacacggcggtattttgggggggagccctcaggctcagggcatattgaccacagtgtcaacaattcctcctcctgcctccaccaatcggcagtcaggaaggcagcctactcccatctctccacctctaagagacagtcatcctcaggccatgcagtggaa

SEQ ID NO: 4 - DNA, 3214 bp, Hepatitis B virus
tccaccactttccaccaaactcttcaagatcccagagtcagggccctgtactttcctgctggtggctccagttcaggaacagtgagccctgctcagactactgtctctgccatatcgtcaatcttatcgaagactggggaccctgtaccgaacatggagaacatcgcatcaggactcctaggacccctgctcgtgttacaggcggggtttttcttgttgacaaaaatcctcacaataccacagagtctagactcgtggtggacttctctcaattttctagggggaamacccgtgtgtcttggccaaaattcgcagtcccaaatctccagtcactcacyaacctgttgtcctccaatttgtcctggttatcgctggatgtgtctgcggcgttttatcatcttcctytgcatcctgctgctatgcctcatcttcttgttggttcttctggactatcraggtatgttgcccgtttgtcctcwamttccaggatcawcaacaaccagcaccggaccatgcaaaacctgcacgactcctgctcaaggaacctctatryktccctcatgttgctgtacaaaacctacggacggaaactgcacctgtattcccatcccatcatcttgggctttcgcaaaatacctatgggagtsggcctcagyccgtttctcttggctcagtttactagcgccatttgttcagtggttcgtagggctttcccccactgtctggctttcagttatatggatgatgtggtattgggggccaagtctgtacaacatcttgagtccctttatgccgctgttaccaatttycttttgtctttgggtatacayttgaaccctcacaaaacaaaaagatggggatattcccttaacttcatgggatatgtaattgggtgttggggcacattgccacaggaacatattgtacaaaaaatcaaaatgtgttttmggaaacttcctgtaaacagacctattgattggaaagtatgtcaacgaattgtgggtcttttggggtttgccgcccctttcacgcaatgtggatatcctgctttratgcctttatatgcatgtatacaagcaaaacaggcttttactttctcgccaacttacaaggcctttctaagtaaacagtatctgaacctttaccccgttactcggcaacggtctggtctgtgccaagtgtttgctgacgcaacccccactggttggggcttggccataggccwtcagcgcatgcgtggaacctttgtgtctcctctgccgatccatactgcggaactcctagccgcttgttttgctcgcagcaggtctggggcaaaactcatcgggactgacaattctgtcgtgctctcccgcaagtatacatcgttcccatggctgctaggctgtgctgccaactggatcctgcgcgggacgtcctttgtttacgtcccgtcggcgctgaatcccgcggacgacccctcccggggccgcttggggctctaccgcccgcttctccgcctgttgtaccgtccgaccacggggcgcacctctctttacgcggactccccgtctgtgccttctcatctrccggaccgtgtgcacttcgcttcacctctgcacgtcgcatggagaccaccgtgaacgcccaccggaacctgcccaaggtcttgcataagaggactcttggactttccgcaatgtcaacgaccgaccttgaggcatacttcaaagactgtgtgtttamtgagtgggaggagttgggggaggagaktaggttaaaggtctttgtactaggaggctgtaggcataaattggtgtgttcaccagcaccatgcaactttttcacctctgcctaatcatctcwtgttcatgtcctactgttcaagcctccaagctgtgccttgggtggctttagggcatggacattgacccgtataaagaatttggagcttctgtggagttactctcttttttgcctmmtgacttctttccttctattcgagatctcctcgacaccgcctctgctttgtatcgggaggccttagagtctccggaacattgttcacctcaccatacggcactcaggcaagctattctgtgttggggtgagttgatgaatctagccacctgggtgggaagtaatttggaagatccagcatccagggaattagtmgttagctatgtcaacgttaatatgggcmtaaaaatcagacaactattgtggtttcacatttcctgtcttacttttgggaragamactgttcttgaatatttggtgtcttttggagtgtggattcgcactcctcctgcatatagaccaycaaatgcccctatcttatcaacacttccggaaactactgttgttagacgaagaggcaggtcccctagaagaagaactccctcgcctcgcagacgaaggtctcaatcgccgcgtcgcagaagatctcaatctcgggaatctcaatgttagtattccttggacacataaggtgggaaactttacggggctttattcttctacggtaccttgctttaatcctaawtggcaaactccttcttttcctgacattcatttgcaggaggacattgttgatagatgtaagcamtttgtggggccccttacagtaaatgaaaacaggagactaaaattaattatgcctgctaggttttatcccaatgttaccaaatatttgcccttagataaagggatcaaaccttattatccagagcatgtagttaatcattacttccagacgagacattatttacayactctttggaaggcgggtatcytatataaaagagagtccacacgtagcgcctcattttgcggatcaccatattcttgggaacaagatctacagcatgggaggttggtcttccaaacctcgaaaaggcatggggacaaatctttctgtccccaatcccctgggattcttcccmgatcatcagttggaccctgcattcaaagccaactcasaaaatccagattgggacctcaacccgcacaaggacaactggccggacgccaacaaggtgggagtgggagcattcgggccagggttcatccctccccatgggggactgttggggtggarccctcaggctcagggcatactcacaactgtgccagcagctcctcctcctgcctccaccaatcggcagtcaggaaggcagcctactcccttatctccacctctaagggacactcatcctcaggccatgcagtggaa

SEQ ID NO: 5 - DNA, 3214 bp, Hepatitis B virus
tccacaacattccaccaagctctgctagatcccagagtgaggggcctatattttcctgctggtggctccagttccggaacagtaaaccctgttccgactactgcctcacccatatcgtcaatcttctcgaggactggggaccctgcaccgaacatggagagcacaacatcaggattcctaggacccctgctcgtgttacaggcggggtttttcttgttgacaagaatcctcacaataccacagagtctagactcgtggtggacttctctcaattttctagggggagcacccacgtgtcctggccaaaattcgcagtccccaacctccaatcactcaccaacctcttgtcctccaatttgtcctggctatcgctggatgtgtctgcggcgttttatcatattcctcttcatcctgctgctatgcctcatcttcttgttggttcttctggactaccaaggtatgttgcccgtttgtcctctacttccaggaacatcaactaccagcacgggaccatgcaagacctgcacgattcctgctcaaggaacctctatgtttccctcttgttgctgtacaaaaccttcggacggaaactgcacttgtattcccatcccatcatcctgggctttcgcaagattcctatgggagtgggccttagtccgtttctcctggctcagtttactagtgccatttgttcagtggttcgcagggctttcccccactgtttggctttcagttatatggatgatgtggtattgggggccaagtctgtacaacatcttgagtccctttttacctctattaccaattttcttttgtcgttgggtatacatttgaaccctaataaaaccaaacgttggggctactcccttaacttcatgggatatgtaattggaagttgggggactttaccacaggaacatattgtattaaaaatcaagcaatgttttcggaaactgcctgtaaatagacctattgattggaaagtatgtcaaagaattgtgggtcttttgggctttgctgccccttttacacaatgtggctatcctgccttgatgcctttatatgcatgtatacaatctaagcaggctttcactttctcgccaacttacaaggcctttctgtgtcaacaatacctgcacctttaccccgttgcccggcaacggtcaggtctctgccaagtgtttgctgacgcaacccccactggatggggcttggccataggccatcggcgcatgcgtggaacctttgtggctcctctgccgatccatactgcggaactcctagcagcttgttttgctcgcagccggtctggagcaaaacttatcgggactgacaactctgttgtcctctctcggaaatacacctccttcccatggctgctcgggtgtgctgccaactggatcctgcgcgggacgtcctttgtctacgtcccgtcggcgctgaatcccgcggacgacccgtctcggggccgtttgggcctctaccgtccccttcttcatctgctgttccagccgactacggggcgcacctctctttacgcggtctccccgtctgtgccttctcatctgccggaccgtgtgcacttcgcttcacctctgcacgtcgcatggagaccaccgtgaatgcccaccaggtcttgcccaagctcttacataagaggactcttggactctcagcaatgtcaacgaccgaccttgaagcatacttcaaagactgtttgtttaaggactgggaggagttgggggaggagattaggttaaaggtctttgtactaggaggctgtaggcataaattggtctgttcaccagcaccatgcaactttttcacctctgcctaatcatctcatgttcatgtcctactgttcaagcctccaagctgtgccttgggtggctttggggcatggacattgacccgtataaagaatttggagcttctgtggagttactctcttttttgccttctgacttctttccttctattcgagatctcctcgacaccgcctctgctctgtatcgggaggccttagagtctccggaacattgttcacctcaccatacagcactcaggcaagctattctctgttggggtgagttgatgaatctggccacctgggtgggaagtaatttggaagacccagcatccagggaattagtagtcagctatgtcaatgttaatatgggcctaaaaatcagacaactattgtggtttcacatttcctgtcttacttttggaagagaaactgttcttgagtatttggtgtcttttggagtgtggattcgcactcctccagcttacagaccaccaaatgcccctatcttatcaacacttccggaaactactgttgttagacgacgaggcaggtcccctagaagaagaactccctcgcctcgcagacgaaggtctcaatcgccgcgtcgcagaagatctcaatctcgggaatctcaatgttagtatcccttggactcataaggtgggaaactttactgggctttattcttctactgttcctgtctttaatcctgagtggcaaactccctcctttcctaacattcatttacaggaagacattattaatagatgtcaacaatatgtgggccctcttacagttaatgaaaaaaggagattaaaattaattatgcctgctaggttctatcctaaccttaccaaatatttgcccttggataaaggcattaaaccttattatcctgaacatgcagttaatcattacttcaaaactaggcattatttacatactctgtggaaggctggcattctatataaaagagaaactacacgcagcgcttcattttgtgggtcaccatattcttgggaacaagagctacagcatgggaggttggtcttccaaacctcgacaaggcatggggacgaatctttctgttcccaatcctctgggattctttcccgatcaccagttggaccctgcgttcggagccaactcaaacaatccagattgggacttcaaccccaacaaggatcactggccagaggcaaatcaggtaggagcgggagcattcgggccagggttcaccccaccacacggcggtcttttggggtggagccctcaggctcagggcatattgacaacagtgccagcagcgcctcctcctgcctccaccaatcggcagtcaggaagacagcctactcccatctctccacctctaagagacagtcatcctcaggccatgcagtggaa

SEQ ID NO: 6 - DNA, 3182 bp, Hepatitis B virus
ttccacaacctttcaccaaactctgcaagatcccagagtgagaggcctgtatttccctgctggtggctccagttcaggagcagtaaaccctgttccgactactgcctctcccttatcgtcaatcttctcgaggattggggaccctgcgctgaacatggagaacatcacatcaggattcctaggaccccttctcgtgttacaggcggggtttttcttgttgacaagaatcctcacaataccgcagagtctagactcgtggtggacttctctcaattttctagggggaactaccgtgtgtcttggccaaaattcgcagtccccaacctccaatcactcaccaacctcctgtcctccaacttgtcctggttatcgctggatgtgtctgcggcgttttatcatcttcctcttcatcctgctgctatgcctcatcttcttgttggttcttctggactatcaaggtatgttgcccgtttgtcctctaattccaggatcctcaaccaccagcacgggaccatgccgaacctgcatgactactgctcaaggaacctctatgtatccctcctgttgctgtaccaaaccttcggacggaaattgcacctgtattcccatcccatcatcctgggctttcggaaaattcctatgggagtgggcctcagcccgtttctcctggctcagtttactagtgccatttgttcagtggttcgtagggctttcccccactgtttggctttcagttatatggatgatgtggtattgggggccaagtctgtacagcatcttgagtccctttttaccgctgttaccaattttcttttgtctttgggtatacatttaaaccctaacaaaacaaagagatggggttactctctgaattttatgggttatgtcattggaagttatgggtccttgccacaagaacacatcatacaaaaaatcaaagaatgttttagaaaacttcctattaacaggcctattgattggaaagtatgtcaacgaattgtgggtcttttgggttttgctgccccatttacacaatgtggttatcctgcgttaatgcccttgtatgcatgtattcaatctaagcaggctttcactttctcgccaacttacaaggcctttctgtgtaaacaatacctgaacctttaccccgttgcccggcaacggccaggtctgtgccaagtgtttgctgacgcaacccccactggctggggcttggtcatgggccatcagcgcgtgcgtggaaccttttcggctcctctgccgatccatactgcggaactcctagccgcttgttttgctcgcagcaggtctggagcaaacattatcgggactgataactctgttgtcctctcccgcaaatatacatcgtatccatggctgctaggctgtgctgccaactggatcctgcgcgggacgtcctttgtttacgtcccgtcggcgctgaatcctgcggacgacccttctcggggtcgcttgagactctctcgtccccttctccgtctgccgttccgaccgaccacggggcgcacctctctttacgcggactccccgtctgtgccttctcatctgccggaccgtgtgcacttcgcttcacctctgcacgtcgcatggagaccaccgtgaacgcccaccgaatgttgcccaaggtcttacataagaggactcttggactctctgcaatgtcaacgaccgaccttgaggcatacttcaaagactgtttgtttaaagactgggaggagttgggggaggagattagattaaaggtctttgtactaggaggctgtaggcataaattggtctgcgcaccggcgccatgcacctttttcacctctgcctaatcatctcttgttcatgtcctactgttcaagcctccaagctgtgccttgggtggctttggggcatggacatcgacccttataaagaatttggagctactgtggagttactctcgtttttgccttctgacttctttccttcagtacgagatcttctagataccgcctcagctctgtatcgggaagccttagagtctcctgagcattgttcacctcaccatactgcactcaggcaagcaattctttgctggggggaactaatgactctagctacctgggtgggtgttaatttggaagatccagcatctagagacctagtagtcagttatgtcaacactaatatgggcctaaagttcaggcaactcttgtggtttcacatttcttgtctcacttttggaagagaaaccgttatagagtatttggtgtctttcggagtgtggattcgcactcctccagcttatagaccaccaaatgcccctatcctatcaacacttccggaaactactgttgttagacgacgaggcaggtcccctagaagaagaactccctcgcctcgcagacgaaggtctcaatcgccgcgtcgcagaagatctcaatctcgggaacctcaatgttagtattccttggactcataaggtggggaactttactggtctttattcttctactgtacctgtctttaatcctcattggaaaacaccatcttttcctaatatacatttacaccaagacattatcaaaaaatgtgaacagtttgtaggcccacttacagttaatgagaaaagaagattgcaattgattatgcctgctaggttttatccaaaggttaccaaatatttaccattggataagggtattaaaccttattatccagaacatctagttaatcattacttccaaactagacactatttacacactctatggaaggcgggtatattatataagagagaaacaacacatagcgcctcattttgtgggtcaccatattcttgggaacaagatctacagcatggggcagaatctttccaccagcaatcctctgggattctttcccgaccaccagttggatccagccttcagagcaaacacagcaaatccagattgggacttcaatcccaacaaggacacctggccagacgccaacaaggtaggagctggagcattcgggctgggtttcactccaccgcacggaggccttttggggtggagctctcaggctcagggcatactacaaactttgccagcaaatccgcctcctgcctccaccaatcgccagacaggaaggcagcctaccccgctgtctccacctttgagaaacactcatcctcaggccatgcagtggaa

SEQ ID NO: 7 - DNA, 3212 bp, Hepatitis B virus
ttccacaacattccaccaagctcascaggatcccagagtaagrggcctgtatyttcctgctggtggctccagttccggaacagtgaaccctgttccgactactgcctcactcatctcgtcaatcttctcgaggattggggaccctgcaccgaacatggaaggcatcacatcaggattcctaggacccctgctcgtgttacaggcggggtttttcttgttgacaaaaatcctcacaataccgcagagtctagactcgtggtggacttctctcaattttcyaggggaagctcccgtgtgtcgtggccaaaattcgcagtycccaacctccaatcactcaccaacctcttgtcctccaatttgtcctggctatcgctggatgtgtctgcggcgttttatcatcttcctcttcatcctgctgctatgcctcatcttcttgttggttcttctggactatcaaggtatgttgcccgtttgtcctctaattccaggatcatcaaccaccagtacgggaccctgccgaacctgcacgactcttgctcaaggaacctctatgtttccctcatgttgctgttcaaaaccttcggacggaaattgcacttgtattcccatcccatcatcatgggctttcggaaaattcctatgggagtgggcctcagcccgtttctcctggctcagtttactagtgccatttgttcagtggttcgccgggctttcccccactgtctggctttcagttatatggatgatgtggtattgggggccaagtctgtacaacatcttgagtccctttatacctctgttaccaattttcttttgtctttgggtatacatttaaatcctaacaaaacaaaaagatggggatattccctaaatttcatgggttatgttattggtagttgggggtcattaccacaggaacacatcagaatgaaaatcaaagactgttttagaaaactccctgttaaccggcctattgattggaaagtatgtcaaagaattgtgggtctcttgggctttgctgccccttttacacaatgtggatatcctgctttaatgcctctgtatgcgtgtattcaatctaagcaggctttcactttctcgccaacttacaaggcctttctgtgtaaacaatacctgaacctttaccccgttgcccggcaacggccaggtctgtgccaagtgtttgctgatgcaacccccactggttggggcttggccataggccatcagcgcatgcgtggaacctttgyggctcctctgccgatccatactgcggaactcctggccgcttgttttgctcgcagcaggtctggagcgaaacttattggaacggataattctgtcgttctctcccggaaatatacatcatttccatggctgctaggctgtgctgccaactggatcctgcgagggacgtcctttgtctacgtcccgtcagcgctgaatcctgcggacgacccgtctcggggtcgcttggggatctatcgtccccttctccgtctgccgttccggccgaccacggggcgcacctctctttacgcggtctccccgtctgtgccttctcatctgccggaccgtgtgcacttcgcttcacctctgcacgtcgcatggaaaccaccgtgaacgcccaccaaatcttgcccaaggtcttatataagaggactcttggactctctgcaatgtcaacgaccgaccttgaggcatacttcaaagactgcttgtttaaagactgggaggagttgggggaggagattagattaatgatctttgtactaggaggctgtaggcataaattggtctgcgcaccagcaccatgcaactttttcacctctgcctaatcatctcttgttcatgtcctactgttcaagcctccaagctgtgccttgggtggctttaggacatggacattgacccttataaagaatttggagctwctgtggagttactctcktttttgcctcatgacttctttccttcaataagagatcttctagataccgccacagctctgtatcgggatgccttagaatctcctgagcattgttcacctcaccacacggcactcaggcaagccattctttgctggggggatgtaatgaatctagctacctgggtgggtgtaaatttggaagatccagcatccagggacctggtagtcggttatgtcaatactaatatgggcctaaagttcagacaattattgtggtttcacacttcctgtctcacttttggaagagaaaccgtcttagagtatttggtgtcttttggagtgtggattcgcactcctccaccttatagaccaccaaatgcccctatcttatcaacacttccggagactactgttgttagacgaagaggcaggtcccctagaagaagaactccctcrcctcgcagacgtagatctcaatcgccgcgtcgcagaagatctcaatctccagcttcccgatgttagtattccttggactcacaaggtgggaaattttacggggctttactcttctactatacctgtctttaatcctaactggaaaactccatcttttcctgatattcatttgcaccaggacattattaacaaatgtgaacaatttgtaggtcccctaacagtaaatgaaaaacgaagattmaacttagtcatgcctgctagattttttcccatctctacgaaatatttgcctctagagaaaggtataaaaccctattatccagataatgtagttaatcattacttccaaaccagacactatttacataccctatggaaggcgggtatcttatataaaagagaaactgcacgtagcgcctcattttgtgggtcaccatattcttgggaacaagagctacatcatgggtctttcttggacggtccctctcgaatgggggaagaatcattccaccaccaatcctctgggattttttcccgaccaccagttggatccagcattcagagcaaacaccagaaatccagattgggaccacaatcccaacaaagaccactggacagaagccaacaaggtaggagtgggagcattcgggccggggttcactcccccacacggaggccttttggggtggagccctcaggctcaaggcatgctaaaaacattgccagcagatccgcctcctgcctccaccaatcggcagtcaggaaggcagcctaccccaatcactccacctttgagagacactcatcctcaggccatrcagtggaa

SEQ ID NO: 8 - DNA, 3205 bp, Hepatitis B virus
ttccatcaggctctgttggatcccagggtaagggctctgtatcttcctgctggtggctccagttcaggaacacaaaaccctgctccgactattgcctctctcacatcctcaatcttctcgacgactgggggccctgctatgaacatggacaacattacatcaggactcctaggacccctgctcgtgttacaggcggtgtgtttcttgttgacaaaaatcctcacaataccacagagtctagactcgtggtggacttctctcaattttctagggggactacccgggtgtcctggccaaaattcgcagtccccaacctccaatcacttaccaacctcctgtcctccaacttgtcctggctatcgttggatgtgtctgcggcgttttatcatcttcctcttcatcctgctgctatgcctcatcttcttgttggttcttctggactaccagggtatgttgcccgtttgtcctctacttccaggatccacgaccaccagcacgggaccctgcaaaacctgcacaactcttgcacaaggaacctctatgtttccctcctgttgctgttcaaaaccctcggacggaaactgcacttgtattcccatcccatcatcctgggctttaggaaaatacctatgggagtgggcctcagcccgtttctcatggctcagtttactagtgcaatttgttcagtggtgcgtagggctttcccccactgtctggcttttagttatattgatgatctggtattgggggccaaatctgtgcagcaccttgagtccctttataccgctgttaccaattttctgttatctgtgggtatccatttaaatacttctaaaactaagagatggggttacaccctacattttatgggttatgtcattggtagttggggatcattacctcaagatcatattgtacacaaaatcaaagaatgttttcggaaactgcctgtaaatcgtccaattgattggaaagtctgtcaacgcattgtgggtcttttgggctttgctgcccctttcacacaatgtggttatcctgctctcatgcctctgtatgcttgtattactgctaaacaggcttttgttttttcgccaacttacaaggcctttctctgtaaacaatacatgaacctttaccccgttgccaggcaacggccgggcctgtgccaagtgtttgctgacgcaacccccactggttggggcttggccattggccatcagcgcatgcgtggaacctttgtggctcctctgccgatccatactgcggaactccttgcagcttgtttcgctcgcagcaggtctggagcgactctcatcggcacggacaactctgttgtcctctctaggaagtacacctccttcccatggctgctcgggtgtgctgcaaactggatcctgcgcgggacgtcctttgtttacgtcccgtcggcgctgaatcccgcggacgacccctcccggggccgcttggggctgtaccgccctcttctccgtctgccgttccagccgacaacgggtcgcacctctctttacgcggactccccgtctgttccttctcatctgccggaccgtgtgcacttcgcttcacctctgcacgtcgcatggagaccaccgtgaacgccccttggagtttgccaacagtcttacataagaggactcttggactttcaggagggtcaatgacccggattgcagaatacatcaaagactgtgtatttaaggactgggaggagttgggggaggagactaggttaatgatctttgtactaggaggctgtaggcataaattggtctgttcaccagcaccatgcaactttttcacctctgcctaatcatcttttgttcatgtcctactgttcaagcctccaagctgtgccttgggtggctttgggacatggacattgacccttataaagaatttggcgcttctgtggagttactctcttttttgccttctgatttctttccatcggttcgggacctactcgacaccgcttcagccctttaccgggatgctttagagtcacctgaacattgcactccccatcacactgccctcaggcaagttattttgtgctggggtgagttaatgactttggcttcctgggtgggcaataacttggaagaccctgctgccagggatttagtagttaactatgttaacactaacatgggcctaaaaattagacaactactgtggtttcacatttcctgccttacttttggaagagatatagttcttgagtatttggtgtcctttggagtgtggattcgcactcctcctgcttacagaccacaaaatgcccctatcctatccacacttccggaaactactgttgttagacgacgaggcaggtcccctagaagaagaactccctcgcctcgcagacgaagatctcaatcgccgcgtcgccgaagatctcaatctccagcttcccaatgttagtattccttggactcataaggtgggaaattttacggggctttactcttctactgtgcctgcttttaatcctgactggttaactccttcttttcctaatattcatttacatcaagacctaatttctaaatgtgaacaatttgtaggcccactcactaaaaatgaattaaggaggttaaaattggttatgccagctagattttatcctaaggttaccaaatattttcctatggagaaaggaatcaagccttattatcctgagcatgcagttaatcattactttaaaacaagacattatttgcatactttatggaaggcgggaattttatataagagagaatccacacgtagcgcatcattttgtgggtcaccatattcctgggaacaagagctacagcatgggagcacctctctcaacgacaagaagaggcatgggacagaatctttctgtgcccaatcctctgggattctttccagaccatcagctggatccgctattcaaagcaaattccagcagtcccgactgggacttcaacacaaacaaggacagttggccaatggcaaacaaggtaggagtgggagcatacggtccagggttcacacccccacacggtggcctgctggggtggagccctcaggcacaaggtatgttaacaaccttgccagcagatccgcctcctgcttccaccaatcggcggtccgggagaaagccaaccccagtctctccacctctaagagacactcatccacaggcaatgcagtggaa

SEQ ID NO: 9 - DNA, 3247 bp, Hepatitis B virus
tctacagcattccaccaagctctacaaaatcccaaagtcaggggcctgtattttcctgctggtggctccagttcagggatagtgaaccctgttccgactattgcctctcacatctcgtcaatcttctccaggattggggaccctgcaccgaacatggagaacatcacatcaggattcctaggacccctgctcgtgttacaggcggggtttttcttgttgacaagaatcctcacaataccgcagaatctagactcgtggtggacttctctcaattttctagggggagtgcccgtgtgtcctggcctaaattcgcagtccccaacctccaatcactcaccaatctcctgtcctccaacttgtcctggctatcgctggatgtgtctgcggcgttttatcatattcctcttcatcctgctgctatgcctcatcttcttgttggttcttctggactatcaaggtatgttgcccgtttgtcctctgattccaggatcctcgaccaccagtacgggaccctgcaaaacctgcacgactcctgctcaaggcaactctatgtatccctcatgttgctgtacaaaaccttcggacggaaattgcacctgtattcccatcccatcatcttgggctttcgcaaaatacctatgggagtgggcctcagtccgtttctcttggctcagtttactagtgccatttgttcagtggttcgtagggctttcccccactgtctggctttcagctatatggatgatgtggtattgggggccaaatctgtacaacatcttgagtccctttataccgctgttaccaattttcttttgtctttgggtatacatctaaaccctaacaaaacaaaaagatggggttattccttaaattttatgggatatgtaattggaagttggggtactttgccacaagaacacatcacacagaaaattaagcaatgttttcggaaactccctgttaacaggccaattgattggaaagtctgtcaacgaataactggtctgttgggtttcgctgctccttttacccaatgtggttaccctgccttaatgcctttatatgcatgtatacaagctaagcaggcttttactttctcgccaacttataaggcctttctctgtaaacaatacatgaacctttaccccgttgctaggcaacggcccggtctgtgccaagtgtttgctgacgcaacccccactggttggggcttggccatcggccatcagcgcatgcgtggaacctttgtggctcctctgccgatccatactgcggaactcctagctgcttgttttgctcgcagccggtctggagcaaaactcattgggactgacaattctgtcgtcctttctcggaaatatacatcctttccatggctgctaggctgtgctgccaactggatccttcgcgggacgtcctttgtttacgtcccgtcagcgctgaatccagcggacgacccctcccggggccgtttggggctctgtcgcccccttctccgtctgccgttcctgccgaccacggggcgcacctctctttacgcggtctccccgtctgttccttctcatctgccggaccgtgtgcacttcgcttcacctctgcacgttacatggaaaccgccatgaacacctctcatcatctgccaaggcagttatataagaggactcttggactgtttgttatgtcaacaaccggggtggagaaatacttcaaggactgtgtttttgctgagtgggaagaattaggcaatgagtccaggttaatgacctttgtattaggaggctgtaggcataaattggtctgcgcaccagcaccatgtaactttttcacctctgcctaatcatctcttgttcatgtcctactgttcaagcctccaagctgtgccttgggtggctttagggcatggatagaacaactttgccatatggcctttttggcttagacattgacccttataaagaatttggagctactgtggagttgctctcgtttttgccttctgactttttcccgtctgttcgtgatcttctcgacaccgcttcagctttgtaccgggaatccttagagtcctctgatcattgttcgcctcaccatacagcactcaggcaagcaatcctgtgctggggtgagttgatgactctagccacctgggtgggtaataatttggaagatccagcatccagagatttggtggtcaattatgttaatactaatatgggtttaaaaatcaggcaactattgtggtttcacatttcctgtcttacttttgggagagaaaccgttcttgagtatttggtgtcttttggagtgtggattcgcactcctcctgcttatagaccaccaaatgcccctatcctatcaacacttccggagactactgttgttagacgaagaggcaggtcccctcgaagaagaactccctcgcctcgcagacgaagatctcaatcgccgcgtcgcagaagatctgcatctccagcttcccaatgttagtattccttggactcacaaggtgggaaactttacggggctgtattcttctactatacctgtctttaatcctgattggcaaactccttcttttccaaatatccatttgcatcaagacattataactaaatgtgaacaatttgtgggccctctcacagtaaatgagaaacgaagattaaaactagttatgcctgccagatttttcccaaactctactaaatatttaccattagacaaaggtatcaaaccgtattatccagaaaatgtagttaatcattacttccagaccagacattatttacataccctttggaaggcgggtattctatataagagagaaacatcccgtagcgcttcattttgtgggtcaccatatacttgggaacaagatctacagcatggggctttcttggacggtccctctcgagtggggaaagaacctttccaccagcaatcctctaggattccttcccgatcaccagttggacccagcattcagagcaaataccaacaatccagattgggacttcaatcccaaaaaggacccttggccagaggccaacaaggtaggagttggagcctatggacccgggttcacccctccacacggaggccttttggggtggagccctcagtctcagggcacactaacaactttgccagcagatccgcctcctgcctccaccaatcgtcagtcagggaggcagccgactcccatctctccaccactaagagacagtcatcctcaggccatgcagtggaa

SEQ ID NO: 10 - DNA, 22 bp, Hepatitis B virus
tgccgatccatactgcggaact

SEQ ID NO: 11 - DNA, 22 bp, Hepatitis B virus
acggctaggtatgacgccttga

SEQ ID NO: 12 - protein, 354 aa, Artificial sequence
  Synthesized
MNTKYNKEFLLYLAGFVDSDGSINASISPRQSFKFKHGLKLRFEVGQKTQHRWFLDKLVDEIGVGYVYDNGSVSVYSLSQIKPLHNFLTQLQPFLKLKQKQANLVLKIIEQLPSAKESPDKFLEVCTWVDQIAALNDSKTRKTTSETVRAVLDSLPGSVGGLSPSQASSAASSASSSPGSGISEALRAGAGSGTGYNKEFLLYLAGFVDGDGSIFASIRPRQHAKFKHDLELCFNVRQKTQRRWFLDKLVDEIGVGYVIDWRGASTYKLSQIKPLHNFLTQLQPFLKLKQKQANLVLKIIEQLPSAKESPDKFLEVCTWVDQIAALNDSKTRKTTSETVRAVLDSLSEKKKSSP

SEQ ID NO: 13 - protein, 354 aa, Artificial sequence
  Synthesized
MNTKYNKEFLLYLAGFVDADGSINASIQPRQSFKFKHSLKLRFEVGQKTQRRWFLDKLVDEIGVGYVYDNGSVSVYSLSQIKPLHNFLTQLQPFLKLKQKQANLVLKIIEQLPSAKESPDKFLEVCTWVDQIAALNDSKTRKTTSETVRAVLDSLPGSVGGLSPSQASSAASSASSSPGSGISEALRAGAGSGTGYNKEFLLYLAGFVDGDGSIFASIRPRQHAKFKHDLELCFNVRQKTQRRWFLDKLVDEIGVGYVLDWRGASTYKLSEIKPLHNFLTQLQPFLKLKQKQANLVLKIIEQLPSAKESPDKFLEVCTWVDQIAALNDSRTRKTTSETVRAVLDSLSEKKKSSP

SEQ ID NO: 14 - protein, 354 aa, Artificial sequence
  Synthesized
MNTKYNKEFLLYLAGFVDGDGSINASIAPRQSFKFKHGLKLRFEVGQKTQRRWFLDKLVDEIGVGYVYDNGSVSVYSLSQIKPLHNFLTQLQPFLKLKQKQANLVLKIIEQLPSAKESPDKFLEVCTWVDQIAALNDSKTRKTTSETVRAVLDSLPGSVGGLSPSQASSAASSASSSPGSGISEALRAGAGSGTGYNKEFLLYLAGFVDSDGSIFASIRPRQMAKFKHDLELCFNVRQKTQRRWFLDKLVDEIGVGYVHDWGSVSTYKLSEIKPLHNFLTQLQPFLKLKQKQANLVLKIIEQLPSAKESPDKFLEVCTWVDQIAALNDSKTRKTTSETVRAVLDSLSEKKKSSP

SEQ ID NO: 15 - protein, 354 aa, Artificial sequence
  Synthesized
MNTKYNKEFLLYLAGFVDGDGSINATIAPRQSFKFKHGLKLRFEVGQKTQRRWFLDKLVDEIGVGYVYDNGSVSVYCLSQIKPLHNFLTQLQPFLKLKQKQANLVLKIIEQLPSAKESPDKFLEVCTWVDQIAALNDSKTRKTTSETVRAVLDSLPGSVGGLSPSQASSAASSASSSPGSGISEALRAGAGSGTGYNKEFLLYLAGFVDGDGSIYASIRPRQHAKFKHDLELIFNVRQLTSRRWFLDKLVDEIGVGYVIDWRGASTYKLSEIKPLHNFLTQLQPFLKLKQKQANLVLKIIEQLPSAKESPDKFLEVCTWVDQIAALNDSKTRKTTSETVRAVLDSLSEKKKSSP

SEQ ID NO: 16 - protein, 354 aa, Artificial sequence
  Synthesized
MNTKYNKEFLLYLAGFVDGDGSINATIAPRQSFKFKHGLKLRFEVGQKTQRRWFLDKLVDEIGVGYVYDNGSVSVYCLSQIKPLHNFLTQLQPFLKLKQKQANLVLKIIEQLPSAKESPDKFLEVCTWVDQIAALNDSKTRKTTSETVRAVLDSLPGSVGGLSPSQASSAASSASSSPGSGISEALRAGAGSGTGYNKEFLLYLAGFVDSDGSIYASIRPRQHAKFKHDLELIFNVRQLTSRRWFLDKLVDEIGVGYVIDWRGASTYKLSEIKPLHNFLTQLQPFLKLKQKQANLVLKIIEQLPSAKESPDKFLEVCTWVDQIAALNDSKTRKTTSETVRAVLDSLSEKKKSSP

SEQ ID NO: 17 - protein, 354 aa, Artificial sequence
  Synthesized
MNTKYNKEFLLYLAGFVDGDGSINAAIAPRQSFKFKHGLKLRFEVGQKTQRRWFLDKLVDEIGVGYVYDNGSVSVYCLSQIKPLHNFLTQLQPFLKLKQKQANLVLKIIEQLPSAKESPDKFLEVCTWVDQIAALNDSKTRKTTSETVRAVLDSLPGSVGGLSPSQASSAASSASSSPGSGISEALRAGAGSGTGYNKEFLLYLAGFVDGDGSIYASIRPRQQSKFKHDLELYFNVRQKTRRRWFLDKLVDEIGVGYVNDWRGTSTYKLSEIKPLHNFLTQLQPFLKLKQKQANLVLKIIEQLPSAKESPDKFLEVCTWVDQIAALNDSKTRKTTSETVRAVLDSLSEKKKSSP

SEQ ID NO: 18 - protein, 147 aa, Artificial sequence
  Synthesized
KEFLLYLAGFVDGDGSIFASIRPRQHAKFKHDLELCFNVRQKTQRRWFLDKLVDEIGVGYVIDWRGASTYKLSQIKPLHNFLTQLQPFLKLKQKQANLVLKIIEQLPSAKESPDKFLEVCTWVDQIAALNDSKTRKTTSETVRAVLD

SEQ ID NO: 19 - protein, 147 aa, Artificial sequence
  Synthesized
KEFLLYLAGFVDGDGSIFASIRPRQHAKFKHDLELCFNVRQKTQRRWFLDKLVDEIGVGYVLDWRGASTYKLSEIKPLHNFLTQLQPFLKLKQKQANLVLKIIEQLPSAKESPDKFLEVCTWVDQIAALNDSRTRKTTSETVRAVLD

SEQ ID NO: 20 - protein, 147 aa, Artificial sequence
  Synthesized
KEFLLYLAGFVDSDGSIFASIRPRQMAKFKHDLELCFNVRQKTQRRWFLDKLVDEIGVGYVHDWGSVSTYKLSEIKPLHNFLTQLQPFLKLKQKQANLVLKIIEQLPSAKESPDKFLEVCTWVDQIAALNDSKTRKTTSETVRAVLD

SEQ ID NO: 21 - protein, 147 aa, Artificial sequence
  Synthesized
KEFLLYLAGFVDGDGSIYASIRPRQHAKFKHDLELIFNVRQLTSRRWFLDKLVDEIGVGYVIDWRGASTYKLSEIKPLHNFLTQLQPFLKLKQKQANLVLKIIEQLPSAKESPDKFLEVCTWVDQIAALNDSKTRKTTSETVRAVLD

SEQ ID NO: 22 - protein, 147 aa, Artificial sequence
  Synthesized
KEFLLYLAGFVDSDGSIYASIRPRQHAKFKHDLELIFNVRQLTSRRWFLDKLVDEIGVGYVIDWRGASTYKLSEIKPLHNFLTQLQPFLKLKQKQANLVLKIIEQLPSAKESPDKFLEVCTWVDQIAALNDSKTRKTTSETVRAVLD

SEQ ID NO: 23 - protein, 147 aa, Artificial sequence
  Synthesized
KEFLLYLAGFVDGDGSIYASIRPRQQSKFKHDLELYFNVRQKTRRRWFLDKLVDEIGVGYVNDWRGTSTYKLSEIKPLHNFLTQLQPFLKLKQKQANLVLKIIEQLPSAKESPDKFLEVCTWVDQIAALNDSKTRKTTSETVRAVLD

SEQ ID NO: 24 - protein, 147 aa, Artificial sequence
  Synthesized
KEFLLYLAGFVDSDGSINASISPRQSFKFKHGLKLRFEVGQKTQHRWFLDKLVDEIGVGYVYDNGSVSVYSLSQIKPLHNFLTQLQPFLKLKQKQANLVLKIIEQLPSAKESPDKFLEVCTWVDQIAALNDSKTRKTTSETVRAVLD

SEQ ID NO: 25 - protein, 147 aa, Artificial sequence
  Synthesized
KEFLLYLAGFVDADGSINASIQPRQSFKFKHSLKLRFEVGQKTQRRWFLDKLVDEIGVGYVYDNGSVSVYSLSQIKPLHNFLTQLQPFLKLKQKQANLVLKIIEQLPSAKESPDKFLEVCTWVDQIAALNDSKTRKTTSETVRAVLD

SEQ ID NO: 26 - protein, 147 aa, Artificial sequence
  Synthesized
KEFLLYLAGFVDGDGSINASIAPRQSFKFKHGLKLRFEVGQKTQRRWFLDKLVDEIGVGYVYDNGSVSVYSLSQIKPLHNFLTQLQPFLKLKQKQANLVLKIIEQLPSAKESPDKFLEVCTWVDQIAALNDSKTRKTTSETVRAVLD

SEQ ID NO: 27 - protein, 147 aa, Artificial sequence
  Synthesized
KEFLLYLAGFVDGDGSINATIAPRQSFKFKHGLKLRFEVGQKTQRRWFLDKLVDEIGVGYVYDNGSVSVYCLSQIKPLHNFLTQLQPFLKLKQKQANLVLKIIEQLPSAKESPDKFLEVCTWVDQIAALNDSKTRKTTSETVRAVLD

SEQ ID NO: 28 - protein, 147 aa, Artificial sequence; identical to SEQ ID NO: 27
  Synthesized

SEQ ID NO: 29 - protein, 147 aa, Artificial sequence
  Synthesized
KEFLLYLAGFVDGDGSINAAIAPRQSFKFKHGLKLRFEVGQKTQRRWFLDKLVDEIGVGYVYDNGSVSVYCLSQIKPLHNFLTQLQPFLKLKQKQANLVLKIIEQLPSAKESPDKFLEVCTWVDQIAALNDSKTRKTTSETVRAVLD

SEQ ID NO: 30 - DNA, 22 bp, Hepatitis B virus
gatgatgtggtattgggggcca

SEQ ID NO: 31 - DNA, 22 bp, Hepatitis B virus
ctactacaccataacccccggt

SEQ ID NO: 32 - DNA, 22 bp, Artificial sequence
  Synthesized
tgccgatccatactgcggaact

SEQ ID NO: 33 - DNA, 19 bp, Artificial sequence
  Synthesized
ggtctgtgccaagtgtttg

SEQ ID NO: 34 - DNA, 20 bp, Artificial sequence
  Synthesized
gtatatttccgcgagaggac

SEQ ID NO: 35 - DNA, 24 bp, Artificial sequence
  Synthesized
cttggcccccaataccacatcatc

SEQ ID NO: 36 - DNA, 23 bp, Artificial sequence
  Synthesized
ggatggaaattgcacctgtattc

SEQ ID NO: 37 - DNA, 24 bp, Artificial sequence
  Synthesized
gggtttaaatgtatacccagagac

SEQ ID NO: 38 - protein, 42 aa, Artificial Sequence
  Synthesized
SLPGSVGGLSPSQASSAASSASSSPGSGISEALRAGAGSGTG

SEQ ID NO: 39 - protein, 354 aa, Artificial Sequence
  Synthesized
MNTKYNKEFLLYLAGFVDGDGSINASIAPRQSFKFKHGLKLRFEVGQKTQRRWFLDKLVDEIGVGYVYDNGSVSVYSLSQIKPLHNFLTQLQPFLKLKQKQANLVLKIIEQLPSAKESPDKFLEVCTWVDQIAALNDSKTRKTTSETVRAVLDSLPGSVGGLSPSQASSAASSASSSPGSGISEALRAGAGSGTGYNKEFLLYLAGFVDGDGSIYASIRPRQYAKFKHDLELRFNVRQKTQRRWFLDKLVDEIGVGYVVDWGSVSTYQLSQIKPLHNFLTQLQPFLKLKQKQANLVLKIIEQLPSAKESPDKFLEVCTWVDQIAALNDSKTRKTTSETVRAVLDSLSEKKKSSP

SEQ ID NO: 40 - protein, 354 aa, Artificial Sequence
  Synthesized
MNTKYNKEFLLYLAGFVDGDGSINAAIAPRQSFKFKHGLKLRFEVGQKTQRRWFLDKLVDEIGVGYVYDNGSVSVYCLSQIKPLHNFLTQLQPFLKLKQKQANLVLKIIEQLPSAKESPDKFLEVCTWVDQIAALNDSKTRKTTSETVRAVLDSLPGSVGGLSPSQASSAASSASSSPGSGISEALRAGAGSGTGYNKEFLLYLAGFVDGDGSIYASIRPRQHAKFKHDLELIFNVRQLTSRRWFLDKLVDEIGVGYVIDWGGASTYKLSEIKPLHNFLTQLQPFLKLKQKQANLVLKIIEQLPSAKESPDKFLEVCTWVDQIAALNDSKTRKTTSETVRAVLDSLSEKKKSSP

SEQ ID NO: 41 - DNA, 22 bp, Hepatitis B virus
cccctgctcgtgttacaggcgg

SEQ ID NO: 42 - DNA, 22 bp, Hepatitis B virus
ggggacgagcacaatgtccgcc

SEQ ID NO: 43 - DNA, 22 bp, Hepatitis B virus
tttgctgacgcaacccccactg

SEQ ID NO: 44 - DNA, 22 bp, Hepatitis B virus
aaacgactgcgttgggggtgac

SEQ ID NO: 45 - DNA, 1065 bp, Artificial sequence
  Synthesized
atgaatacaaaatataataaagagttcttactctacttagcagggtttgtagactctgacggttccatcaacgccagcatctcgccgcggcagtcgttcaagttcaagcacgggctgaagctccggttcgaggtcggtcagaagacacagcaccgttggttcctcgacaagctggtggacgagatcggtgtgggttacgtgtatgacaatggcagcgtctccgtttactctctgtcccagatcaagcctttgcataattttttaacacaactacaaccttttctaaaactaaaacaaaaacaagcaaatttagttttaaaaattattgaacaacttccgtcagcaaaagaatccccggacaaattcttagaggtttgtacatgggtggatcaaattgcagctctgaatgattcgaagacgcgtaaaacaacttctgaaaccgttcgtgctgtgctagacagtttaccaggatccgtgggaggtctatcgccatctcaggcatccagcgccgcatcctcggcttcctcaagcccgggttcagggatctccgaagcactcagagctggagcaggttccggcactggatacaacaaggaattcctgctctacctggcgggcttcgtcgacggggacggctccatctttgcatcgatccggcctcgtcaacatgctaagttcaagcacgatctggagctctgtttcaatgtcaggcagaagacacagcgccgttggttcctcgacaagctggtggacgagatcggtgtgggttacgtgattgactggcgtggcgcctccacttacaagctgtcccagatcaagcctctgcacaacttcctgacccagctccagcccttcctgaagctcaagcagaagcaggccaacctcgtgctgaagatcatcgagcagctgccctccgccaaggaatccccggacaagttcctggaggtgtgcacctgggtggaccagatcgccgctctgaacgactccaagacccgcaagaccacttccgaaaccgtccgcgccgttctagacagtctctccgagaagaagaagtcgtccccctaa

SEQ ID NO: 46 - DNA, 1065 bp, Artificial sequence
  Synthesized
atgaatacaaaatataataaagagttcttactctacttagcagggtttgtagacgctgacggttccatcaacgccagcatccagccgcggcagtcgttcaagttcaagcactctctgaagctccggttcgaggtcggtcagaagacacagcgccgttggttcctcgacaagctggtggacgagatcggtgtgggttacgtgtatgacaatggcagcgtctccgtttactctctgtcccagatcaagcctttgcataattttttaacacaactacaaccttttctaaaactaaaacaaaaacaagcaaatttagttttaaaaattattgaacaacttccgtcagcaaaagaatccccggacaaattcttagaagtttgtacatgggtggatcaaattgcagctctgaatgattcgaagacgcgtaaaacaacttctgaaaccgttcgtgctgtgctagacagtttaccaggatccgtgggaggtctatcgccatctcaggcatccagcgccgcatcctcggcttcctcaagcccgggttcagggatctccgaagcactcagagctggagcaggttccggcactggatacaacaaggaattcctgctctacctggcgggcttcgtcgacggggacggctccatctttgcatcgatccggcctcgtcaacatgctaagttcaagcacgatctggagctctgtttcaatgtcaggcagaagacacagcgccgttggttcctcgacaagctggtggacgagatcggtgtgggttacgtgcttgactggcgtggcgcctccacttacaagctgtccgagatcaagcctctgcacaacttcctgacccagctccagcccttcctgaagctcaagcagaagcaggccaacctcgtgctgaagatcatcgagcagctgccctccgccaaggaatccccggacaagttcctggaggtgtgcacctgggtggaccagatcgccgctctgaacgactccaggacccgcaagaccacttccgaaaccgtccgcgccgttctagacagtctctccgagaagaagaagtcgtccccctaa

SEQ ID NO: 47 - DNA, 1065 bp, Artificial sequence
  Synthesized
atgaatacaaaatataataaagagttcttactctacttagcagggtttgtagacggtgacggttccatcaatgccagtatcgctccgcggcagtcgtttaagttcaagcacggtctgaagctccggttcgaggtcggtcagaagacacagcgccgttggttcctcgacaagctggtggacgagatcggtgtgggttacgtgtatgacaatggcagcgtctccgtttactctctgtcccagatcaagcctttgcataattttttaacacaactacaaccttttctaaaactaaaacaaaaacaagcaaatttagttttaaaaattattgaacaacttccgtcagcaaaagaatccccggacaaattcttagaagtttgtacatgggtggatcaaattgcagctctgaatgattcgaagacgcgtaaaacaacttctgaaaccgttcgtgctgtgctagacagtttaccaggatccgtgggaggtctatcgccatctcaggcatccagcgccgcatcctcggcttcctcaagcccgggttcagggatctccgaagcactcagagctggagcaggttccggcactggatacaacaaggaattcctgctctacctggcgggcttcgtcgactccgacggctccatctttgcatcgatccggcctcgtcaaatggctaagttcaagcacgatctggagctctgtttcaatgtcaggcagaagacacagcgccgttggttcctcgacaagctggtggacgagatcggtgtgggttacgtgcatgactggggcagcgtctccacttacaagctgtccgagatcaagcctctgcacaacttcctgacccagctccagcccttcctgaagctcaagcagaagcaggccaacctcgtgctgaagatcatcgagcagctgccctccgccaaggaatccccggacaagttcctggaggtgtgcacctgggtggaccagatcgccgctctgaacgactccaagacccgcaagaccacttccgaaaccgtccgcgccgttctagacagtctctccgagaagaagaagtcgtccccctaa

SEQ ID NO: 48 - DNA, 1065 bp, Artificial sequence
  Synthesized
atgaatacaaaatataataaagagttcttactctacttagcagggtttgtagacggtgacggttccatcaatgccactatcgctccgcggcagtcgtttaagttcaagcacggtctgaagctccggttcgaggtcggtcagaagacacagcgccgttggttcctcgacaagctggtggacgagatcggtgtgggttacgtgtatgacaatggcagcgtctccgtttactgtctgtcccagatcaagcctttgcataattttttaacacaactacaaccttttctaaaactaaaacaaaaacaagcaaatttagttttaaaaattattgaacaacttccgtcagcaaaagaatccccggacaaattcttagaagtttgtacatgggtggatcaaattgcagctctgaatgattcgaagacgcgtaaaacaacttctgaaaccgttcgtgctgtgctagacagtttaccaggatccgtgggaggtctatcgccatctcaggcatccagcgccgcatcctcggcttcctcaagcccgggttcagggatctccgaagcactcagagctggagcaggttccggcactggatacaacaaggaattcctgctctacctggcgggcttcgtcgacggggacggctccatctatgcatctatcaggcctcgtcaacatgctaagttcaagcacgatctggagctcattttcaatgtcaggcagctgacaagccgccgttggttcctcgacaagctggtggacgagatcggtgtgggttacgtgattgactggcgtggcgcctccacttacaagctgtccgagatcaagcctctgcacaacttcctgacccagctccagcccttcctgaagctcaagcagaagcaggccaacctcgtgctgaagatcatcgagcagctgccctccgccaaggaatccccggacaagttcctggaggtgtgcacctgggtggaccagatcgccgctctgaacgactccaagacccgcaagaccacttccgaaaccgtccgcgccgttctagacagtctctccgagaagaagaagtcgtccccctaa

SEQ ID NO: 49 - DNA, 1065 bp, Artificial sequence
  Synthesized
atgaatacaaaatataataaagagttcttactctacttagcagggtttgtagacggtgacggttccatcaatgccactatcgctccgcggcagtcgtttaagttcaagcacggtctgaagctccggttcgaggtcggtcagaagacacagcgccgttggttcctcgacaagctggtggacgagatcggtgtgggttacgtgtatgacaatggcagcgtctccgtttactgtctgtcccagatcaagcctttgcataattttttaacacaactacaaccttttctaaaactaaaacaaaaacaagcaaatttagttttaaaaattattgaacaacttccgtcagcaaaagaatccccggacaaattcttagaagtttgtacatgggtggatcaaattgcagctctgaatgattcgaagacgcgtaaaacaacttctgaaaccgttcgtgctgtgctagacagtttaccaggatccgtgggaggtctatcgccatctcaggcatccagcgccgcatcctcggcttcctcaagcccgggttcagggatctccgaagcactcagagctggagcaggttccggcactggatacaacaaggaattcctgctctacctggcgggcttcgtcgactccgacggctccatctatgcatctatcaggcctcgtcaacatgctaagttcaagcacgatctggagctcattttcaatgtcaggcagctgacaagccgccgttggttcctcgacaagctggtggacgagatcggtgtgggttacgtgattgactggcgtggcgcctccacttacaagctgtccgagatcaagcctctgcacaacttcctgacccagctccagcccttcctgaagctcaagcagaagcaggccaacctcgtgctgaagatcatcgagcagctgccctccgccaaggaatccccggacaagttcctggaggtgtgcacctgggtggaccagatcgccgctctgaacgactccaagacccgcaagaccacttccgaaaccgtccgcgccgttctagacagtctctccgagaagaagaagtcgtccccctaa

SEQ ID NO: 50 - DNA, 1065 bp, Artificial sequence
  Synthesized
atgaatacaaaatataataaagagttcttactctacttagcagggtttgtagacggtgacggttccatcaatgccgcgatcgctccgcggcagtcgtttaagttcaagcacggtctgaagctccggttcgaggtcggtcagaagacacagcgccgttggttcctcgacaagctggtggacgagatcggtgtgggttacgtgtatgacaatggcagcgtctccgtttactgtctgtcccagatcaagcctttgcataattttttaacacaactacaaccttttctaaaactaaaacaaaaacaagcaaatttagttttaaaaattattgaacaacttccgtcagcaaaagaatccccggacaaattcttagaagtttgtacatgggtggatcaaattgcagctctgaatgattcgaagacgcgtaaaacaacttctgaaaccgttcgtgctgtgctagacagtttaccaggatccgtgggaggtctatcgccatctcaggcatccagcgccgcatcctcggcttcctcaagcccgggttcagggatctccgaagcactcagagctggagcaggttccggcactggatacaacaaggaattcctgctctacctggcgggcttcgtcgacggggacggctccatctatgcaagtatcaggcctcgtcaacagtcgaagttcaagcacgatctggagctctatttcaatgtcaggcagaagacaaggcgccgttggttcctcgacaagctggtggacgagatcggtgtgggttacgtgaatgactggcgtggcacctccacttacaagctgtccgagatcaagcctctgcacaacttcctgacccagctccagcccttcctgaagctcaagcagaagcaggccaacctcgtgctgaagatcatcgagcagctgccctccgccaaggaatccccggacaagttcctggaggtgtgcacctgggtggaccagatcgccgctctgaacgactccaagacccgcaagaccacttccgaaaccgtccgcgccgttctagacagtctctccgagaagaagaagtcgtccccctaa

SEQ ID NO: 51 - protein, 10 aa, Artificial Sequence
  Synthesized
MAPKKKRKVH